European Patent Specification EP 3 423 483 B1, published September 24, 2025. Title: HUMAN KYNURENINASE ENZYME VARIANTS HAVING IMPROVED PHARMACOLOGICAL PROPERTIES. Applicant: Board of Regents, the University of Texas System. The sequence listing filed with the application follows.

SEQUENCE LISTING (34 sequences)

SEQ ID NO: 1 - protein, 465 aa, Homo sapiens
MEPSSLELPADTVQRIAAELKCHPTDERVALHLDEEDKLRHFRECFYIPKIQDLPPVDLSLVNKDENAIYFLGNSLGLQPKMVKTYLEEELDKWAKIAAYGHEVGKRPWITGDESIVGLMKDIVGANEKEIALMNALTVNLHLLMLSFFKPTPKRYKILLEAKAFPSDHYAIESQLQLHGLNIEESMRMIKPREGEETLRIEDILEVIEKEGDSIAVILFSGVHFYTGQHFNIPAITKAGQAKGCYVGFDLAHAVGNVELYLHDWGVDFACWCSYKYLNAGAGGIAGAFIHEKHAHTIKPALVGWFGHELSTRFKMDNKLQLIPGVCGFRISNPPILLVCSLHASLEIFKQATMKALRKKSVLLTGYLEYLIKHNYGKDKAATKKPVVNIITPSHVEERGCQLTITFSVPNKDVFQELEKRGVVCDKRNPNGIRVAPVPLYNSFHDVYKFTNLLTSILDSAETKN

SEQ ID NO: 2 - protein, 465 aa, Artificial sequence
  Synthetic polypeptide
MEPSSLELPADTVQRIAAELKCHPTDERVALHLDEEDKLRHFRECFYIPKIQDLPPVDLSLVNKDENAIYFLGNSLGLQPKMVKTYLEEELDKWAKIAIYGHEVGKRPWITADESIVGLMKDIVGANEKEIALMNALTVNLHLLMLSFFKPTPKRYKILLEAKAFPSDHYAIESQLQLHGLNIEESMRMIKPREGEETLRIEDILEVIEKEGDSIAVILFSGVHFYTGQHFNIPAITKAGQAKGCYVGFDLAHAVGNVELYLHDWGVDFACWCSYKYLNAGAGGIAGAFIHEKHAHTIKPALVGWYGHELSTRFKMDNKLQLIPGVCGFRNSNPPILLVCSLHASLEIFKQATMKALRKKSVLLTGYLEYLIKHNYGKDKAATKKPVVNIITPSHVEERGCQLTLTFNVPNKDVFQELEKRGVVCDKRNPNGIRVTPVPLYNSFHDVYKFTNLLTSILDSAETKN

SEQ ID NO: 3 - protein, 465 aa, Artificial sequence
  Synthetic polypeptide
MEPSSLELPADTVQRIAAELKCHPTDERVALHLDEEDKLRHFRECFYIPKIQDLPPVDLSLVNKDENAIYFLGNSLGLQPKMVKTYLEEELDKWAKIAIYGHEVGKRPWITADESIVGLMKDIVGANEKEIALMNALTVNLHLLMLSFFKPTPKRYKILLEAKAFPSDHYAIESQLQLHGLNIEESMRMIEPREGEETLRIEDILEVIEKEGDSIAVILFSGVHFYTGQHFNIPAITKAGQAKGCYVGFDLAHAVGNVELYLHDWGVDFACWCSYKYLNAGAGGIAGAFIHEKHAHTIKPALVGWYGHELSTRFKMDNKLQLIPGVCGFRISNPPILLVCSLHASLEIFKQATMKALRKKSVLLTGYLEYLIKHNYGKDKSATKKPVVNIITPSHVEERGCQLTLTFNVPNKDVFQELEKRGVVCDKRNPNGIRVTPVPLYNSFHDVYKFTNLLTSILDSAETKN

SEQ ID NO: 4 - protein, 465 aa, Artificial sequence
  Synthetic polypeptide
MEPSSLELPADTVRRIAAELKCHPTDERVALHLDEEDKLRHFRECFYIPKIQDLPPVDLSLVNKDENAIYFLGNSLGLQPKMVKTYLEEELDKWAKIAIYGHEVGKRPWITADESIVGLMKDIVGANEKEIALMNALTVNLHLLMLSFFKPTPKRYKILLEAKAFPSDHYAIESQLQLHGLNIEESMRIIKPREGEETLRIEDILEVIEKEGDSIAVILFSGVHFYTGQYFNIPAITKAGQAKGCYVGFDLAHAVGNVELYLHDWGVDFACWCSYKYLNAGAGGIAGAFIHEKHAHTIKPALVGWYGHELSTRFKMDNKLQLIPGVCGFRNSNPPILLVCSLHASLEIFKQATMKALRKKSVLLTGYLEYLIKHNYGKDKAATKKPVVNIITPSHVEERGCQLTLTFNVPNKDVFQELEKRGVVCDKRNPNGIRVTPVPLYNSFHDVYKFTNLLTSILDSAETKN

SEQ ID NO: 5 - protein, 465 aa, Artificial sequence
  Synthetic polypeptide
MEPSSLELPADTVQRIAAELKCHPTDERVALHLDEEDKLRHFRECFYIPKIQDLPPVDLSLVNKDENAIYFLGNSLGLQPKMVKTYLEEELDKWAKIAAYGHEVGKRPWITGDESIVGLMKDIVGANEKEIALMNALSVNLHLLMLSFFKPTPKRYKILLEAKAFPSDHYAIESQLQLHGLNIEESMRMIKPREGEETLRIEDILEVIEKEGDSIAVILFSGVNYYTGQHFNIPAITKAGQAKGCYVGFDLAHAVGNVELYLHDWGVDFACWCSYKYLNAGAGGIAGAFIHEKHAHTIKPALVGWWGHELSTRFKMDNKLQLIPGVCGFRISTPPILLVCSLHASLEIFKQATMKALRKKSVLLTGYLEYLIKHNYGKDKAATKKPVVNIITPSHVEERGCQLTITFNVPNKDVFQELEKRGVVCDKRNPNGIRVTPVPLYNSFHDVYKFTNLLTSILDSAETKN

SEQ ID NO: 6 - protein, 465 aa, Artificial sequence
  Synthetic polypeptide
MEPSSLELPADTVQRIAAELKCHPTDERVALHLDEEDKLRHFRECFYIPKIQDLPPVDLSLVNKDEDAIYFNGNSLGLQPKMVKTYLEEELDKWAKIAAYGHQVGKRPWITGDESIVGLMKDIVGANEKEIALMNALTVNLHLLMLSFFKPTPKRYKILLEAKAFPSDHYAIESQLQLHGLNIEESMRMIKPREGEETLRIEDILEVIEKEGDSIAVILFSGVHYYTGQHFNIPAITKAGQAKGCYVGFDLAHAVGNVELYLHDWGVDFACWCSYKYLNAGAGGIAGAFIHEKHAHTIKPALVGWFGHELSTRFKMDNKLQLIPGVCGFRVSNPPILLVCSLHASLEIFKQATMKALRKKSVLLTGYLEYLIKHNYGKDKAATKKPVVNIITPSHVEERGCQLTITFNVPNKDVFQELEKRGVVCDKRNPNGIRVTPVPLYNSFHDVYKFTNLLTSILDSAETKN

SEQ ID NO: 7 - protein, 465 aa, Artificial sequence
  Synthetic polypeptide
MEPSSLELPADTVQRIAAELKCHPTDERVALHLDEEDKLRHFRECFYIPKIQDLPPVDLSLVNKDEDAIYFLGNSLGLQPKMVKTYLEEELDKWAKIAAYGHEVGKRPWITGDESIVGLMKDIVGANEKEIALMNSLSVNLHLLMLSFFKPTPKRYKILLEAKAFPSDHYAIESQLQLHGLNIEESMRMIKPREGEETLRIEDILEVIEKEGDSIAVILFSGVHYYTGQHFNIPAITKAGQAKGCYVGFDLAHAVGNVELYLHDWGVDFACWCSYKYLNAGAGGIAGAFIHEKHAHTIKPALVGWFGHELSTRFKMDNKLQLIPGVCGFRISNPPILLVCSLHASLEIFKQATMKALRKKSVLLTGYLEYLIKHNYGKDKAATKKPVVNIITPSHVEERGCQLTITFNVPNKDVFQELEKRGVVCDKRNPNGIRVTPVPLYNSFHDVYKFTNLLTSILDSAETKN

SEQ ID NO: 8 - protein, 465 aa, Artificial sequence
  Synthetic polypeptide
MEPSSLELPADTVQRIAAELKCHPTDERVALHLDEEDKLRHFRECFYIPKIQDLPPVDLSLVNKDENAIYFLGNSLGLQPKMVKTYLEEELDKWAKIASYGHEVGKRPWITGDESIVGLMKDIVGANEKEIALMNGTTVNLHLLMLSFFKPTPKRYKILLEAKAFPSDHYAIESQLQLHGLNIEESMRMIKPREGEETLRIEDILEVIEKEGDSIAVILFSGVHFYTGQHFNIPAITKAGQAKGCYVGFDLAHAVGNVELYLHDWGVDFACWCSYKYLNAGAGGIAGAFIHEKHAHTIKPALVGWLGHELSTRFKMDNKLQLIPGVCGFRISNPPILLVCSLHASLEIFKQATMKALRKKSVLLTGYLEYLIKHNYGKDKAATKKPVVNIITPSHVEERGCQLTITFSVPNKDVFQELEKRGVVCDKRNPNGIRVTPVPLYNSFHDVYKFTNLLTSILDSAETKN

SEQ ID NO: 9 - DNA, 4719 bp, Escherichia coli
ccgacaccatcgaatggtgcaaaacctttcgcggtatggcatgatagcgcccggaagagagtcaattcagggtggtgaatgtgaaaccagtaacgttatacgatgtcgcagagtatgccggtgtctcttatcagaccgtttcccgcgtggtgaaccaggccagccacgtttctgcgaaaacgcgggaaaaagtggaagcggcgatggcggagctgaattacattcccaaccgcgtggcacaacaactggcgggcaaacagtcgttgctgattggcgttgccacctccagtctggccctgcacgcgccgtcgcaaattgtcgcggcgattaaatctcgcgccgatcaactgggtgccagcgtggtggtgtcgatggtagaacgaagcggcgtcgaagcctgtaaagcggcggtgcacaatcttctcgcgcaacgcgtcagtgggctgatcattaactatccgctggatgaccaggatgccattgctgtggaagctgcctgcactaatgttccggcgttatttcttgatgtctctgaccagacacccatcaacagtattattttctcccatgaagacggtacgcgactgggcgtggagcatctggtcgcattgggtcaccagcaaatcgcgctgttagcgggcccattaagttctgtctcggcgcgtctgcgtctggctggctggcataaatatctcactcgcaatcaaattcagccgatagcggaacgggaaggcgactggagtgccatgtccggttttcaacaaaccatgcaaatgctgaatgagggcatcgttcccactgcgatgctggttgccaacgatcagatggcgctgggcgcaatgcgcgccattaccgagtccgggctgcgcgttggtgcggatatctcagtagtgggatacgacgataccgaagacagctcatgttatatcccgccgttaaccaccatcaaacaggattttcgcctgctggggcaaaccagcgtggaccgcttgctgcaactctctcagggccaggcggtgaagggcaatcagctgttgcccgtctcactggtgaaaagaaaaaccaccctggcgcccaatacgcaaaccgcctctccccgcgcgttggccgattcattaatgcagctggcacgacaggtttcccgactggaaagcgggcagtgagcgcaacgcaattaatgtaagttagctcactcattaggcacaattctcatgtttgacagcttatcatcgactgcacggtgcaccaatgcttctggcgtcaggcagccatcggaagctgtggtatggctgtgcaggtcgtaaatcactgcataattcgtgtcgctcaaggcgcactcccgttctggataatgttttttgcgccgacatcataacggttctggcaaatattctgaaatgagctgttgacaattaatcatcggctcgtataatgtgtggaattgtgagcggataacaatttcacacaggaaacagccagtccgtttaggtgttttcacgagcacttcaccaacaagtggtacctaatgcattgataaaaccgcgcgaaggtgaggagaccctgcggattgaggacatcctggaggtgatcgagaaggagggcgacagtatcgcggtgatacttttcagcggcgtgcatttctacacgggccaacacttcaatatcccggccattaccaaagccggccaggcgaaagggtgctatgtaggctttgatctggcgcatgcagtgggcaacgtcgaactgtatcttcatgattggggcgttgattttgcgtgctgccgcggattacccgggctgcaggcaagcttggcactggccgtcgttttacaacgtcgtgactgggaaaaccctggcgttacccaacttaatcgccttgcagcacatccccatttcgccagctggcgtaatagcgaagaggcccgcaccgatcgcccttcccaacagttgcgcagcctgaatggcgaatggcagcttggctgttttggcggatgagataagattttcagcctgatacagattaaatcagaacgcagaagcggtctgataaaacagaatttgcctggcggcagtagcgcggtggtcccacctgaccccatgccgaactcagaagtgaaacgccgtagcgccgatggtagtgtggggtctccccatgcgagagtagggaactgccaggcatcaaataaaacgaaaggctcagtcgaaagactgggcctttcgttttatctgttgtttgtcggtgaacgctctcctgagtaggacaaatccgccgggagcggatttgaacgttgcgaagcaacggcccggagggtggcgggcaggacgcccgccataaactgccaggcatcaaattaagcagaaggccatcctgacggatggcctttttaacgtttacaatttcaggtggcacttttcggggaaatgtgcgcggaacccctatttgtttatttttctaaatacattcaaatatgtatccgctcatgtcgagacgttgggtgaggttccaactttcaccataatgaaataagatcactaccgggcgtattttttgagttatcgagattttcaggagctaaggaagctaaaatggagaaaaaaatcactggatataccaccgttgatatatcccaatggcatcgtaaagaacattttgaggcatttcagtcagttgctcaatgtacctataaccagaccgttcagctggatattacggcctttttaaagaccgtaaagaaaaataagcacaagttttatccggcctttattcacattcttgcccgcctgatgaatgctcatccggagttccgtatggcaatgaaagacggtgagctggtgatatgggatagtgttcacccttgttacaccgttttccatgagcaaactgaaacgttttcatcgctctggagtgaataccacgacgatttccggcagtttctacacatatattcgcaagatgtggcgtgttacggtgaaaacctggcctatttccctaaagggtttattgagaatatgtttttcgtctcagccaatccctgggtgagtttcaccagttttgatttaaacgtggccaatatggacaacttcttcgcccccgttttcaccatgggcaaatattatacgcaaggcgacaaggtgctgatgccgctggcgattcaggttcatcatgccgtttgtgatggcttccatgtcggcagaatgcttaatgaattacaacagtactgcgatgagtggcagggcggggcgtaatttttttaaggcagttattggtgcccttaaacgcctggttgctacgcctgaataagtgataataagcggatgaatggcagaaattcgaaagcaaattcgacccggtcgtcggttcagggcagggtcgttaaatagccgcttatgtctattgctggtttaccggtttattgactaccggaagcagtgtgaccgtgtgcttctcaaatgcctgaggccagtttgctcaggctctccccgtggaggtaataattaaaaggatctaggtgaagatcctttttgataatctcatgaccaaaatcccttaacgtgagttttcgttccactgagcgtcagaccccgtagaaaagatcaaaggatcttcttgagatcctttttttctgcgcgtaatctgctgcttgcaaacaaaaaaaccaccgctaccagcggtggtttgtttgccggatcaagagctaccaactctttttccgaaggtaactggcttcagcagagcgcagataccaaatactgtccttctagtgtagccgtagttaggccaccacttcaagaactctgtagcaccgcctacatacctcgctctgctaatcctgttaccagtggctgctgccagtggcgataagtcgtgtcttaccgggttggactcaagacgatagttaccggataaggcgcagcggtcgggctgaacggggggttcgtgcacacagcccagcttggagcgaacgacctacaccgaactgagatacctacagcgtgagctatgagaaagcgccacgcttcccgaagggagaaaggcggacaggtatccggtaagcggcagggtcggaacaggagagcgcacgagggagcttccagggggaaacgcctggtatctttatagtcctgtcgggtttcgccacctctgacttgagcgtcgatttttgtgatgctcgtcaggggggcggagcctatggaaaaacgccagcaacgcggcctttttacggttcctggccagttaagccagtatacactccgctatcgctacgtgactgggtcatggctgcgccccgacacccgccaacacccgctgacgcgccctgacgggcttgtctgctcccggcatccgcttacagacaagctgtgaccgtctccgggagctgcatgtgtcagaggttttcaccgtcatcaccgaaacgcgcgaggcagctgcggtaaagctcatcagcgtggtcgtgcagcgattcacagatgtctgcctgttcatccgcgtccagctcgttgagtttctccagaagcgttaatgtctggcttctgataaagcgggccatgttaagggcggttttttcctgtttggtcactgatgcctccgtgtaagggggatttctgttcatgggggtaatgataccgatgaaacgagagaggatgctcacgatacgggttactgatgatgaacatgcccggttactggaacgttgtgagggtaaacaactggcggtatgg

SEQ ID NO: 10 - DNA, 39 bp, Artificial sequence
  Synthetic primer
taaacaactggcggtatggccgacaccatcgaatggtgc

SEQ ID NO: 11 - DNA, 50 bp, Artificial sequence
  Synthetic primer
gttttatcaatgcattaggtaccacttgttggtgaagtgctcgtgaaaac

SEQ ID NO: 12 - DNA, 40 bp, Artificial sequence
  Synthetic primer
gtgtatactggcttaactggccaggaaccgtaaaaaggcc

SEQ ID NO: 13 - DNA, 52 bp, Artificial sequence
  Synthetic primer
ataggccgaaatcggcaaaaggatctaggtgaagatcctttttgataatctc

SEQ ID NO: 14 - DNA, 48 bp, Artificial sequence
  Synthetic primer
ctttttacggttcctggccagttaagccagtatacactccgctatcgc

SEQ ID NO: 15 - DNA, 42 bp, Artificial sequence
  Synthetic primer
accattcgatggtgtcggccataccgccagttgtttaccctc

SEQ ID NO: 16 - DNA, 38 bp, Artificial sequence
  Synthetic primer
tgccgcggattacccgggctgcaggcaagcttggcact

SEQ ID NO: 17 - DNA, 42 bp, Artificial sequence
  Synthetic primer
cacctgaaattgtaaacgttaaaaaggccatccgtcaggatg

SEQ ID NO: 18 - DNA, 47 bp, Artificial sequence
  Synthetic primer
ctgacggatggcctttttaacgtttacaatttcaggtggcacttttc

SEQ ID NO: 19 - DNA, 46 bp, Artificial sequence
  Synthetic primer
gatcttcacctagatccttttaattattacctccacggggagagcc

SEQ ID NO: 20 - DNA, 37 bp, Artificial sequence
  Synthetic primer
gtggtacctaatgcattgataaaaccgcgcgaaggtg

SEQ ID NO: 21 - DNA, 38 bp, Artificial sequence
  Synthetic primer
agcccgggtaatccgcggcagcacgcaaaatcaacgcc

SEQ ID NO: 22 - protein, 465 aa, Artificial sequence
  Synthetic polypeptide
MEPSSLELPADTVQRIAAELKCHPTDERVALHLDEEDKLRHFRECFYIPKIQDLPPVDLSLVNKDENAIYFLGNSLGLQPKMVKTYLEEELDKWAKIAIYGHEVGKRPWITADESIVGLMKDIVGANEKEIALMNALTVNLHLLMLSFFKPTPKRYKILLEAKAFPSDHYAIESQLQLHGLNIEESMRMIKPREGEETLRIEDILEVIEKEGDSIAVILFSGVHFYTGQHFNIPAITKAGQAKGCYVGFDLAHAVGNVELYLHDWGVDFACWCSYKYLNAGAGGIAGAFIHEKHAHTIKPALVGWYGHELSTRFKMDNKLQLIPGVCGFRISNPPILLVCSLHASLEIFKQATMKALRKKSVLLTGYLEYLIKHNYGKDKAATKKPVVNIITPSHVEERGCQLTLTFNVPNKDVFQELEKRGVVCDKRNPNGIRVTPVPLYNSFHDVYKFTNLLTSILDSAETKN

SEQ ID NO: 23 - DNA, 53 bp, Artificial sequence
  Synthetic primer
cactgtgtggtaccgaggtaatacatgggcggtcatcatcaccaccatcatgg

SEQ ID NO: 24 - DNA, 50 bp, Artificial sequence
  Synthetic primer
cgagtcagcccgggtaatccgcggctagtttttggtttccgcactgtcca

SEQ ID NO: 25 - DNA, 1347 bp, Artificial sequence
  Synthetic oligonucleotide
tctagaaataattttgtttaactttaaggaaaacattaaaataaggaggtagcaaatgggcggtcatcatcaccaccatcatgggagcggcaccacccgcaacgattgcctggcgctggatgcgcaggatagcctggcaccgctgcgtcagcagtttgcgctgccggaaggtgttatttatctggatggcaacagcctgggtgcgcgtccggttgcggcgctggcgcgtgcgcaggcggtgattgcggaagaatggggcaacggcctgattcgcagctggaacagcgcgggctggcgcgatctgagcgaacgcctgggcaaccgcctggcgaccctgattggcgcgcgcgatggcgaagtggtggtgaccgataccaccagcattaacctgtttaaagtgctgagcgcggcgctgcgcgtgcaggcgacccgcagcccggaacgccgcgtgattgtgaccgaaaccagcaactttccgaccgatctgtatattgcggaaggcctggcggatatgctgcagcagggctataccctgcgcctggtggatagcccggaagaactgccgcaggcgattgatcaggataccgcggtggtgatgctgacccatgtgaactataaaaccggctatatgcatgatatgcaggcgctgaccgcgctgagccatgaatgcggcgcgctggcgatttgggatctggcgcatagcgcgggcgcggtgccggtggatctgcatcaggcgggcgcggattatgcgattggctgcacctataaatatctgaacggcggcccgggcagccaggcgtttgtgtgggtgagcccgcagctgtgcgatctggtgccgcagccgctgtctggttggtttggccatagccgccagtttgcgatggaaccgcgctatgaaccgagcaacggcattgcgcgctatctgtgcggcacccagccgattaccagcctggcgatggtggaatgcggcctggatgtgtttgcgcagaccgatatggcgagcctgcgccgcaaaagcctggcgctgaccgatctgtttattgaactggtggaacagcgctgcgcggcgcatgaactgaccctggtgaccccgcgcgaacatgcgaaacgcggcagccatgtgagctttgaacatccggaaggctatgcggtgattcaggcgctgattgatcgcggcgtgattggcgattatcgcgaaccgcgcattatgcgctttggctttaccccgctgtataccacctttaccgaagtgtgggatgcggtgcagattctgggcgaaattctggatcgcaaaacctgggcgcaggcgcagtttcaggtgcgccatagcgtgacctagtaggatcc

SEQ ID NO: 26 - protein, 465 aa, Artificial sequence
  Synthetic polypeptide
MEPSSLELPADTVQRIAAELKCHPTDERVALHLDEEDKLRHFRECFYIPKIQDLPPVDLSLVNKDENAIYFLGNSLGLQPKMVKTYLEEELDKWAKIASYGHEVGKRPWITGDESIVGLMKDIVGANEKEIALMNALTVNLHLLMLSFFKPTPKRYKILLEAKAFPSDHYAIESQLQLHGLNIEESMRMIKPREGEETLRIEDILEVIEKEGDSIAVILFSGVHFYTGQHFNIPAITKAGQAKGCYVGFDLAHAVGNVELYLHDWGVDFACWCSYKYLNAGAGGIAGAFIHEKHAHTIKPALVGWLGHELSTRFKMDNKLQLIPGVCGFRISNPPILLVCSLHASLEIFKQATMKALRKKSVLLTGYLEYLIKHNYGKDKAATKKPVVNIITPSHVEERGCQLTITFSVPNKDVFQELEKRGVVCDKRNPNGIRVTPVPLYNSFHDVYKFTNLLTSILDSAETKN

SEQ ID NO: 27 - DNA, 1398 bp, Artificial sequence
  Synthetic oligonucleotide
atggaaccgagctcccttgaacttccggccgataccgtgcaacggatagcggcggaattgaaatgtcacccgaccgacgaacgcgtcgcgttacatctggatgaggaagacaagctgcgtcacttccgcgagtgcttttacattccgaaaattcaggatctgccgccagtggacttgagcctggtcaacaaagacgagaacgccatctacttcctgggcaatagcctgggcctgcaaccaaagatggtgaaaacctatcttgaggaggagcttgacaaatgggcgaagatcgcgatctacggccatgaagtcggcaagcgtccctggattaccgctgatgagtcaatcgttggcttgatgaaggatatcgtcggcgcgaacgagaaagaaattgcgctgatgaacgcgctgaccgtgaatctgcatctgctgatgctgtcattctttaagcccaccccgaagcgctacaaaatcctgctggaagcgaaagcgtttcccagcgatcattatgcgatagaaagccagctgcaactgcacggcctgaatatcgaggagagcatgcgtatgataaaaccgcgcgaaggtgaggagaccctgcggattgaggacatcctggaggtgatcgagaaggagggcgacagtatcgcggtgatacttttcagcggcgtgcatttctacacgggccaacacttcaatatcccggccattaccaaagccggccaggcgaaagggtgctatgtaggctttgatctggcgcatgcagtgggcaacgtcgaactgtatcttcatgattggggcgttgattttgcgtgctggtgcagctataagtatctgaatgccggggccggtgggattgcgggagcctttattcatgagaaacacgcgcataccattaaaccggcgctggttggctggtatgggcacgaactgagcacccgcttcaagatggataacaaactgcaattgattccgggcgtgtgcggctttcgtaatagcaaccccccgattctgctggtctgcagcctgcacgcgtctctggagattttcaagcaggcgaccatgaaagcgctgcgtaagaaaagtgtgcttctgacgggctacctggagtacctgataaagcacaactacggcaaggataaggcggccacgaagaagccggttgtgaacattatcaccccgtctcatgtggaagaacgtggctgccaactgacgcttacgttcaacgtgccaaacaaggacgtgttccaagagctggagaagcgtggcgtggtgtgtgataaacgtaatccgaatggcattcgtgtgacgcctgtgccgctgtacaacagcttccacgacgtgtataagttcaccaacctgctgacgagcattctggacagtgcggaaaccaaaaactag

SEQ ID NO: 28 - DNA, 1398 bp, Artificial sequence
  Synthetic oligonucleotide
atggaaccgagctcccttgaacttccggccgataccgtgcaacggatagcggcggaattgaaatgtcacccgaccgacgaacgcgtcgcgttacatctggatgaggaagacaagctgcgtcacttccgcgagtgcttttacattccgaaaattcaggatctgccgccagtggacttgagcctggtcaacaaagacgagaacgccatctacttcctgggcaatagcctgggcctgcaaccaaagatggtgaaaacctatcttgaggaggagcttgacaaatgggcgaagatcgcgatctacggccatgaagtcggcaagcgtccctggattaccgctgatgagtcaatcgttggcttgatgaaggatatcgtcggcgcgaacgagaaagaaattgcgctgatgaacgcgctgaccgtgaatctgcatctgctgatgctgtcattctttaagcccaccccgaagcgctacaaaatcctgctggaagcgaaagcgtttcccagcgatcattatgcgatagaaagccagctgcaactgcacggcctgaatatcgaggagagcatgcgtatgatagaaccgcgcgaaggtgaggagaccctgcggattgaggacatcctggaggtgatcgagaaggagggcgacagtatcgcggtgatacttttcagcggcgtgcatttctacacgggccaacacttcaatatcccggccattaccaaagccggccaggcgaaagggtgctatgtaggctttgatctggcgcatgcagtgggcaacgtcgaactgtatcttcatgattggggcgttgattttgcgtgctggtgcagctataagtatctgaatgccggggccggtgggattgcgggagcctttattcatgagaaacacgcgcataccattaaaccggcgctggttggctggtatgggcacgaactgagcacccgcttcaagatggataacaaactgcaattgattccgggcgtgtgcggctttcgtattagcaaccccccgattctgctggtctgcagcctgcacgcgtctctggagattttcaagcaggcgaccatgaaagcgctgcgtaagaaaagtgtgcttctgacgggctacctggagtacctgataaagcacaactacggcaaggataagtcggccacgaagaagccggttgtgaacattatcaccccgtctcatgtggaagaacgtggctgccaactgacgcttacgttcaacgtgccaaacaaggacgtgttccaagagctggagaagcgtggcgtggtgtgtgataaacgtaatccgaatggcattcgtgtgacgcctgtgccgctgtacaacagcttccacgacgtgtataagttcaccaacctgctgacgagcattctggacagtgcggaaaccaaaaactag

SEQ ID NO: 29 - DNA, 1398 bp, Artificial sequence
  Synthetic oligonucleotide
atggaaccgagctcccttgaacttccggccgataccgtgcgacggatagcggcggaattgaaatgtcacccgaccgacgaacgcgtcgcgttacatctggacgaggaagacaagctgcgtcacttccgcgagtgcttttacattccgaaaattcaggatctgccgccagtggacttgagcctggtcaacaaagacgagaacgccatctacttcctgggtaatagcctgggcctgcaaccaaagatggtgaaaacctatcttgaggaggagcttgacaaatgggcgaagatcgcgatctacggccatgaagtcggcaagcgtccctggattaccgctgatgagtcaatcgttggcttgatgaaggatatcgtcggcgcgaacgagaaagaaattgcgctgatgaacgcgctgaccgtgaatctgcatctgctgatgctgtcattctttaagcccaccccgaagcgctacaaaatcctgctggaagcgaaagcgtttcccagcgatcattatgcgatagaaagccagctgcaactgcacggcctgaatatcgaggagagcatgcgtataataaaaccgcgcgaaggtgaggagaccctgcggattgaggacatcctggaggtgatcgagaaggagggcgacagtatcgcggtgatacttttcagcggcgtgcatttctacacgggccaatacttcaatatcccggccattaccaaagctggccaggcgaaagggtgctatgtaggctttgatctggcgcatgcagtgggcaacgtcgaactgtatcttcatgattggggcgttgattttgcgtgctggtgcagctataagtatctgaatgccggggccggtgggattgcgggagcctttattcatgagaaacatgcgcataccattaaaccggcgctggttggctggtatgggcacgaactgagcacccgcttcaagatggataacaaactgcaattgattccgggcgtgtgcggctttcgtaatagcaaccccccgattctgctggtctgcagcctgcacgcgtctctggagattttcaagcaggcgactatgaaagcgctgcgtaagaaaagtgtgcttctgacgggctatctggagtacctgataaagcacaactacggcaaggataaggcggccacgaagaagccggttgtgaacattatcaccccgtctcatgtggaagaacgtggctgccaactgacgcttacgttcaacgtgccaaacaaggacgtgttccaagagctggagaagcgtggcgtggtgtgtgataaacgtaatccgaatggcattcgtgtgacgcctgtgccgctgtacaacagcttccacgacgtgtataagttcaccaacctgctgacgagcattctggacagtgcggaaaccaaaaactag

SEQ ID NO: 30 - DNA, 1398 bp, Artificial sequence
  Synthetic oligonucleotide
atggaaccgagctcccttgaacttccggccgataccgtgcaacggatagcggcggaattgaaatgtcacccgaccgacgaacgcgtcgcgttacatctggatgaggaagacaagctgcgtcacttccgcgagtgcttttacattccgaaaattcaggatctgccgccagtggacttgagcctggtcaacaaagacgagaatgccatctatttcctgggcaatagcctgggcctgcaaccaaagatggtgaaaacctatcttgaggaggagcttgacaaatgggcgaagatcgcggcctacggccatgaggtcggcaagcgtccctggattaccggcgatgagtcaatcgttggcttgatgaaggatatcgtcggcgcgaacgagaaagaaattgcgctgatgaacgccttatctgtgaatctgcatctgctgatgctgtcattctttaagcccaccccgaagcgctacaaaatcctgctggaagcgaaagcgtttcccagcgatcattatgcgatagaaagccagctgcaactgcacggcctgaatatcgaggagagcatgcgtatgataaaaccgcgcgaaggtgaggagaccctgcggattgaggacatcctggaggtgatcgagaaggagggcgacagtatcgcggtgatacttttctctggcgtgaattattacacgggccaacacttcaatatcccggccattaccaaagccggccaggcgaaagggtgctatgtaggctttgatctggcgcatgcagtgggcaacgtcgaactgtatcttcatgattggggcgttgattttgcgtgctggtgcagctataagtatctgaatgccggggccggtgggattgcgggagcctttattcatgagaaacacgcgcataccattaaaccggcgctggttggctggtgggggcacgaactgagcacccgcttcaagatggataacaaactgcaattgattccgggcgtgtgcggctttcgtattagcaccccgccgattctgctggtctgcagcctgcacgcgtctctggagattttcaagcaggcgaccatgaaagcgctgcgtaagaaaagtgtgcttctgacgggctacctggagtacctgataaagcacaactacggcaaggataaggcggccacgaagaagccggttgtgaacattatcaccccgtctcatgtggaagaacgtggctgccagctgacgataacgttcaacgtgccaaacaaggacgtgttccaagagctggagaagcgtggcgtggtgtgtgataaacgtaatccgaatggcattcgtgtgacgcctgtgccgctgtacaacagcttccacgacgtgtataagttcaccaacctgctgacgagcattctggacagtgcggaaaccaaaaactag

SEQ ID NO: 31 - DNA, 1398 bp, Artificial sequence
  Synthetic oligonucleotide
atggaaccgagctcccttgaacttccggccgataccgtgcaacggatagcggcggaattgaaatgtcacccgaccgacgaacgcgtcgcgttacatctggatgaggaagacaagctgcgtcacttccgcgagtgcttttacattccgaaaattcaggatctgccgccagtggacttgagcctggtcaacaaagacgaggatgccatctatttcaatggcaatagcctgggcctgcaaccaaagatggtgaaaacctatcttgaggaggagcttgacaaatgggcgaagatcgcggcctacggccatcaggtcggcaagcgtccctggattaccggcgatgagtcaatcgttggcttgatgaaggatatcgtcggcgcgaacgagaaagaaattgcgctgatgaacgccttaactgtgaatctgcatctgctgatgctgtcattctttaagcccaccccgaagcgctacaaaatcctgctggaagcgaaagcgtttcccagcgatcattatgcgatagaaagccagctgcaactgcacggcctgaatatcgaggagagcatgcgtatgataaaaccgcgcgaaggtgaggagaccctgcggattgaggacatcctggaggtgatcgagaaggagggcgacagtatcgcggtgatacttttctctggcgtgcattattacacgggccaacacttcaatatcccggccattaccaaagccggccaggcgaaagggtgctatgtaggctttgatctggcgcatgcagtgggcaacgtcgaactgtatcttcatgattggggcgttgattttgcgtgctggtgcagctataagtatctgaatgccggggccggtgggattgcgggagcctttattcatgagaaacacgcgcataccattaaaccggcgctggttggctggtttgggcacgaactgagcacccgcttcaagatggataacaaactgcaattgattccgggcgtgtgcggctttcgtgttagcaacccgccgattctgctggtctgcagcctgcacgcgtctctggagattttcaagcaggcgaccatgaaagcgctgcgtaagaaaagtgtgcttctgacgggctacctggagtacctgataaagcacaactacggcaaggataaggcggccacgaagaagccggttgtgaacattatcaccccgtctcatgtggaagaacgtggctgccagctgacgataacgttcaacgtgccaaacaaggacgtgttccaagagctggagaagcgtggcgtggtgtgtgataaacgtaatccgaatggcattcgtgtgacgcctgtgccgctgtacaacagcttccacgacgtgtataagttcaccaacctgctgacgagcattctggacagtgcggaaaccaaaaactag

SEQ ID NO: 32 - DNA, 1398 bp, Artificial sequence
  Synthetic oligonucleotide
atggaaccgagctcccttgaacttccggccgataccgtgcaacggatagcggcggaattgaaatgtcacccgaccgacgaacgcgtcgcgttacatctggatgaggaagacaagctgcgtcacttccgcgagtgcttttacattccgaaaattcaggatctgccgccagtggacttgagcctggtcaacaaagacgaggatgccatctatttcctgggcaatagcctgggcctgcaaccaaagatggtgaaaacctatcttgaggaggagcttgacaaatgggcgaagatcgcggcctacggccatgaggtcggcaagcgtccctggattaccggcgatgagtcaatcgttggcttgatgaaggatatcgtcggcgcgaacgagaaagaaattgcgctgatgaactccttatctgtgaatctgcatctgctgatgctgtcattctttaagcccaccccgaagcgctacaaaatcctgctggaagcgaaagcgtttcccagcgatcattatgcgatagaaagccagctgcaactgcacggcctgaatatcgaggagagcatgcgtatgataaaaccgcgcgaaggtgaggagaccctgcggattgaggacatcctggaggtgatcgagaaggagggcgacagtatcgcggtgatacttttctctggcgtgcattattacacgggccaacacttcaatatcccggccattaccaaagccggccaggcgaaagggtgctatgtaggctttgatctggcgcatgcagtgggcaacgtcgaactgtatcttcatgattggggcgttgattttgcgtgctggtgcagctataagtatctgaatgccggggccggtgggattgcgggagcctttattcatgagaaacacgcgcataccattaaaccggcgctggttggctggtttgggcacgaactgagcacccgcttcaagatggataacaaactgcaattgattccgggcgtgtgcggctttcgtattagcaacccgccgattctgctggtctgcagcctgcacgcgtctctggagattttcaagcaggcgaccatgaaagcgctgcgtaagaaaagtgtgcttctgacgggctacctggagtacctgataaagcacaactacggcaaggataaggcggccacgaagaagccggttgtgaacattatcaccccgtctcatgtggaagaacgtggctgccagctgacgataacgttcaacgtgccaaacaaggacgtgttccaagagctggagaagcgtggcgtggtgtgtgataaacgtaatccgaatggcattcgtgtgacgcctgtgccgctgtacaacagcttccacgacgtgtataagttcaccaacctgctgacgagcattctggacagtgcggaaaccaaaaactag

SEQ ID NO: 33 - DNA, 1398 bp, Artificial sequence
  Synthetic oligonucleotide
atggaaccgagctcccttgaacttccggccgataccgtgcaacggatagcggcggaattgaaatgtcacccgaccgacgaacgcgtcgcgttacatctggatgaggaagacaagctgcgtcacttccgcgagtgcttttacattccgaaaattcaggatctgccgccagtggacttgagcctggtcaacaaagacgagaacgccatctacttcctgggcaatagcctgggcctgcaaccaaagatggtgaaaacctatcttgaggaggagcttgacaaatgggcgaagatcgcgagctacggccatgaagtcggcaagcgtccctggattaccggcgatgagtcaatcgttggcttgatgaaggatatcgtcggcgcgaacgagaaagaaattgcgctgatgaacggcacgaccgtgaatctgcatctgctgatgctgtcattctttaagcccaccccgaagcgctacaaaatcctgctggaagcgaaagcgtttcccagcgatcattatgcgatagaaagccagctgcaactgcacggcctgaatatcgaggagagcatgcgtatgataaaaccgcgcgaaggtgaggagaccctgcggattgaggacatcctggaggtgatcgagaaggagggcgacagtatcgcggtgatacttttcagcggcgtgcatttctacacgggccaacacttcaatatcccggccattaccaaagccggccaggcgaaagggtgctatgtaggctttgatctggcgcatgcagtgggcaacgtcgaactgtatcttcatgattggggcgttgattttgcgtgctggtgcagctataagtatctgaatgccggggccggtgggattgcgggagcctttattcatgagaaacacgcgcataccattaaaccggcgctggttggctggctggggcacgaactgagcacccgcttcaagatggataacaaactgcaattgattccgggcgtgtgcggctttcgtattagcaaccccccgattctgctggtctgcagcctgcacgcgtctctggagattttcaagcaggcgaccatgaaagcgctgcgtaagaaaagtgtgcttctgacgggctacctggagtacctgataaagcacaactacggcaaggataaggcggccacgaagaagccggttgtgaacattatcaccccgtctcatgtggaagaacgtggctgccaactgacgataacgttcagcgtgccaaacaaggacgtgttccaagagctggagaagcgtggcgtggtgtgtgataaacgtaatccgaatggcattcgtgtgacgcctgtgccgctgtacaacagcttccacgacgtgtataagttcaccaacctgctgacgagcattctggacagtgcggaaaccaaaaactag

SEQ ID NO: 34 - DNA, 1497 bp, Artificial sequence
  Synthetic oligonucleotide
tctagaaataattttgtttaactttaaggacaaatcaggacacagttaaggaggtaaaatatgggcggtcatcatcaccaccatcatgggagcggcgaaccgagctcccttgaacttccggccgataccgtgcaacggatagcggcggaattgaaatgtcacccgaccgacgaacgcgtcgcgttacatctggatgaggaagacaagctgcgtcacttccgcgagtgcttttacattccgaaaattcaggatctgccgccagtggacttgagcctggtcaacaaagacgagaacgccatctacttcctgggcaatagcctgggcctgcaaccaaagatggtgaaaacctatcttgaggaggagcttgacaaatgggcgaagatcgcggcctacggccatgaagtcggcaagcgtccctggattaccggcgatgagtcaatcgttggcttgatgaaggatatcgtcggcgcgaacgagaaagaaattgcgctgatgaacgcgctgaccgtgaatctgcatctgctgatgctgtcattctttaagcccaccccgaagcgctacaaaatcctgctggaagcgaaagcgtttcccagcgatcattatgcgatagaaagccagctgcaactgcacggcctgaatatcgaggagagcatgcgtatgataaaaccgcgcgaaggtgaggagaccctgcggattgaggacatcctggaggtgatcgagaaggagggcgacagtatcgcggtgatacttttcagcggcgtgcatttctacacgggccaacacttcaatatcccggccattaccaaagccggccaggcgaaagggtgctatgtaggctttgatctggcgcatgcagtgggcaacgtcgaactgtatcttcatgattggggcgttgattttgcgtgctggtgcagctataagtatctgaatgccggggccggtgggattgcgggagcctttattcatgagaaacacgcgcataccattaaaccggcgctggttggctggtttgggcacgaactgagcacccgcttcaagatggataacaaactgcaattgattccgggcgtgtgcggctttcgtattagcaaccccccgattctgctggtctgcagcctgcacgcgtctctggagattttcaagcaggcgaccatgaaagcgctgcgtaagaaaagtgtgcttctgacgggctacctggagtacctgataaagcacaactacggcaaggataaggcggccacgaagaagccggttgtgaacattatcaccccgtctcatgtggaagaacgtggctgccaactgacgataacgttcagcgtgccaaacaaggacgtgttccaagagctggagaagcgtggcgtggtgtgtgataaacgtaatccgaatggcattcgtgtggcgcctgtgccgctgtacaacagcttccacgacgtgtataagttcaccaacctgctgacgagcattctggacagtgcggaaaccaaaaactagggatcc